European Patent Specification EP 3 521 437 B1, published January 15, 2025. Title: METHODS AND COMPOSITIONS FOR TARGETED GENETIC MODIFICATION USING PAIRED GUIDE RNAS. Applicant: Frendewey, David Lai, Ka-Man Venus Auerbach, Wojtek Lee, Jeffrey D. Mujica, Alexander O. Droguett, Gustavo Trzaska, Sean Hunt, Charleen Gagliardi, Anthony Valenzuela, David M. Voronina, Vera Macdonald, Lynn Murphy, Andrew J. Yancopoulos, George D. The sequence listing filed with the application follows.

SEQUENCE LISTING (176 sequences)

SEQ ID NO: 1 - RNA, 80 nt, Artificial Sequence
  gRNA
guuuuagagcuagaaauagcaaguuaaaauaaggcuaguccguuaucaacuugaaaaaguggcaccgagucggugcuuuu

SEQ ID NO: 2 - RNA, 42 nt, Artificial Sequence
  gRNA
guuuuagagcuagaaauagcaaguuaaaauaaggcuaguccg

SEQ ID NO: 3 - RNA, 30 nt, Artificial Sequence
  crRNA
guuuuagagcuagaaauagcaaguuaaaau

SEQ ID NO: 4 - RNA, 33 nt, Artificial Sequence
  crRNA
guuuuagagcuagaaauagcaaguuaaaauaag

SEQ ID NO: 5 - RNA, 26 nt, Artificial Sequence
  crRNA
gaguccgagcagaagaagaaguuuua

SEQ ID NO: 6 - RNA, 12 nt, Artificial Sequence
  tracrRNA
aaggcuaguccg

SEQ ID NO: 7 - RNA, 50 nt, Artificial Sequence
  tracrRNA
aaggcuaguccguuaucaacuugaaaaaguggcaccgagucggugcuuuu

SEQ ID NO: 8 - DNA, 23 bp, Artificial Sequence
  CRISPR RNA recognition sequence
  misc_feature (2)...(21): n = a, t, c, or g
gnnnnnnnnnnnnnnnnnnnngg

SEQ ID NO: 9 - DNA, 23 bp, Artificial Sequence
  CRISPR RNA recognition sequence
  misc_feature (1)...(21): n = a, t, c, or g
nnnnnnnnnnnnnnnnnnnnngg

SEQ ID NO: 10 - DNA, 25 bp, Artificial Sequence
  CRISPR RNA recognition sequence
  misc_feature (3)...(23): n = a, t, c, or g
ggnnnnnnnnnnnnnnnnnnnnngg

SEQ ID NO: 11 - DNA, 20 bp, Artificial Sequence
  C5 (Hc) gRNA A DNA-targeting segment
atcacaaaccagttaaccgg

SEQ ID NO: 12 - DNA, 20 bp, Artificial Sequence
  C5 (Hc) gRNA B DNA-targeting segment
tttcagacgagccgacccgg

SEQ ID NO: 13 - DNA, 20 bp, Artificial Sequence
  C5 (Hc) gRNA C DNA-targeting segment
tgtgtgtcatagcgatgtcg

SEQ ID NO: 14 - DNA, 20 bp, Artificial Sequence
  C5 (Hc) gRNA D DNA-targeting segment
aacaggtaccctatcctcac

SEQ ID NO: 15 - DNA, 20 bp, Artificial Sequence
  C5 (Hc) gRNA E DNA-targeting segment
ggcccggacctagtctctct

SEQ ID NO: 16 - DNA, 20 bp, Artificial Sequence
  C5 (Hc) gRNA E2 DNA-targeting segment
tcgtggttgcatgcgcactg

SEQ ID NO: 17 - DNA, 20 bp, Artificial Sequence
  Lrp5 gRNA A DNA-targeting segment
gggaacccacagcatactcc

SEQ ID NO: 18 - DNA, 20 bp, Artificial Sequence
  Lrp5 gRNA B DNA-targeting segment
gaatcatgcacggctacccc

SEQ ID NO: 19 - DNA, 20 bp, Artificial Sequence
  Lrp5 gRNA B2 DNA-targeting segment
tgctcctatggggaggcgcg

SEQ ID NO: 20 - DNA, 20 bp, Artificial Sequence
  Lrp5 gRNA C DNA-targeting segment
actgagatcaatgaccccga

SEQ ID NO: 21 - DNA, 20 bp, Artificial Sequence
  Lrp5 gRNA D DNA-targeting segment
gggtcgcccggaacctctac

SEQ ID NO: 22 - DNA, 20 bp, Artificial Sequence
  Lrp5 gRNA E2 DNA-targeting segment
cttggataacattgataccc

SEQ ID NO: 23 - DNA, 20 bp, Artificial Sequence
  Lrp5 gRNA E DNA-targeting segment
ggggcagagcccttatatca

SEQ ID NO: 24 - DNA, 20 bp, Artificial Sequence
  Lrp5 gRNA F DNA-targeting segment
tcgctcacattaatccctag

SEQ ID NO: 25 - DNA, 20 bp, Artificial Sequence
  Ror1 gRNA A DNA-targeting segment
tgtgggcctttgctgatcac

SEQ ID NO: 26 - DNA, 20 bp, Artificial Sequence
  Ror1 gRNA B DNA-targeting segment
aatctatgatcctatggcct

SEQ ID NO: 27 - DNA, 20 bp, Artificial Sequence
  Ror1 gRNA D DNA-targeting segment
tgccaatagcagtgacttga

SEQ ID NO: 28 - DNA, 20 bp, Artificial Sequence
  Ror1 gRNA C DNA-targeting segment
gggaagaatgggctattgtc

SEQ ID NO: 29 - DNA, 20 bp, Artificial Sequence
  Ror1 gRNA E DNA-targeting segment
ggttgtttgtgctgatgacg

SEQ ID NO: 30 - DNA, 20 bp, Artificial Sequence
  Ror1 gRNA F DNA-targeting segment
ccgtcctaggccttctacgt

SEQ ID NO: 31 - DNA, 20 bp, Artificial Sequence
  Trpa1 gRNA A DNA-targeting segment
gtactggggaatcggtggtc

SEQ ID NO: 32 - DNA, 20 bp, Artificial Sequence
  Trpa1 gRNA A2 DNA-targeting segment
cacgcactccaaatttatcc

SEQ ID NO: 33 - DNA, 20 bp, Artificial Sequence
  Trpa1 gRNA B DNA-targeting segment
ctaagtgtgtatcagtacat

SEQ ID NO: 34 - DNA, 20 bp, Artificial Sequence
  Trpa1 gRNA C DNA-targeting segment
tgccctgcacaataagcgca

SEQ ID NO: 35 - DNA, 20 bp, Artificial Sequence
  Trpa1 gRNA D DNA-targeting segment
actcattgaaacgttatggc

SEQ ID NO: 36 - DNA, 20 bp, Artificial Sequence
  Trpa1 gRNA E2 DNA-targeting segment
agtaagggtggattaaattc

SEQ ID NO: 37 - DNA, 20 bp, Artificial Sequence
  Trpa1 gRNA E DNA-targeting segment
gccatctagattcatgtaac

SEQ ID NO: 38 - DNA, 20 bp, Artificial Sequence
  Trpa1 gRNA F DNA-targeting segment
gactagaaatgttctgcacc

SEQ ID NO: 39 - DNA, 21 bp, Artificial Sequence
  190045 forward primer
gagctcatagccaacagcttg

SEQ ID NO: 40 - DNA, 20 bp, Artificial Sequence
  190061 forward primer
atgcatcagatcacgctcag

SEQ ID NO: 41 - DNA, 20 bp, Artificial Sequence
  190068 forward primer
gtccttgtggcatttccaac

SEQ ID NO: 42 - DNA, 24 bp, Artificial Sequence
  190030 forward primer
ccagtatggtgtcagttaatagcg

SEQ ID NO: 43 - DNA, 19 bp, Artificial Sequence
  190033 forward primer
ctgtgcagaaagcagcctc

SEQ ID NO: 44 - DNA, 20 bp, Artificial Sequence
  190013 forward primer
cctctccctctaggcacctg

SEQ ID NO: 45 - DNA, 20 bp, Artificial Sequence
  190045 reverse primer
tctttaagggctccgttgtc

SEQ ID NO: 46 - DNA, 20 bp, Artificial Sequence
  190061 reverse primer
aagaccaaccattcacccag

SEQ ID NO: 47 - DNA, 20 bp, Artificial Sequence
  190068 reverse primer
ttcccagtccaagtcaaagg

SEQ ID NO: 48 - DNA, 20 bp, Artificial Sequence
  190030 reverse primer
ctgttatctgcaaggcaccc

SEQ ID NO: 49 - DNA, 20 bp, Artificial Sequence
  190033 reverse primer
acaactggatcctgattcgc

SEQ ID NO: 50 - DNA, 20 bp, Artificial Sequence
  190013 reverse primer
taagagggcatgggtgagac

SEQ ID NO: 51 - DNA, 20 bp, Artificial Sequence
  C2 probe (B6)
aattcagaagacctatcgta

SEQ ID NO: 52 - DNA, 21 bp, Artificial Sequence
  T3 probe (B6)
tatgtgtataggtgtttggat

SEQ ID NO: 53 - DNA, 19 bp, Artificial Sequence
  T6 probe (B6)
tacattgctaaatgaaacc

SEQ ID NO: 54 - DNA, 16 bp, Artificial Sequence
  T7 probe (B6)
cgcagtcatgcacata

SEQ ID NO: 55 - DNA, 20 bp, Artificial Sequence
  T8 probe (B6)
ttataaagcccagtatgtac

SEQ ID NO: 56 - DNA, 14 bp, Artificial Sequence
  T9 probe (B6)
tgctgcataatcag

SEQ ID NO: 57 - DNA, 18 bp, Artificial Sequence
  T10 probe (B6)
tcaggagtgaattggata

SEQ ID NO: 58 - DNA, 16 bp, Artificial Sequence
  T11 probe (B6)
ctgctacttacctttg

SEQ ID NO: 59 - DNA, 13 bp, Artificial Sequence
  T13 probe (B6)
aggaggaaaacgc

SEQ ID NO: 60 - DNA, 17 bp, Artificial Sequence
  T14 probe (B6)
cctttgttcctcataag

SEQ ID NO: 61 - DNA, 20 bp, Artificial Sequence
  C2 probe (129)
aattcagaagacctattgta

SEQ ID NO: 62 - DNA, 21 bp, Artificial Sequence
  T3 probe (129)
tatgtgtataggtgtttgcat

SEQ ID NO: 63 - DNA, 16 bp, Artificial Sequence
  T6 probe (129)
cattgctacatgaaac

SEQ ID NO: 64 - DNA, 16 bp, Artificial Sequence
  T7 probe (129)
cgcagtcatgcacgta

SEQ ID NO: 65 - DNA, 23 bp, Artificial Sequence
  T8 probe (129)
tgagaatttataaagcccaatat

SEQ ID NO: 66 - DNA, 14 bp, Artificial Sequence
  T9 probe (129)
tgctgcatgatcag

SEQ ID NO: 67 - DNA, 15 bp, Artificial Sequence
  T10 probe (129)
tcaggagtgaatcgg

SEQ ID NO: 68 - DNA, 16 bp, Artificial Sequence
  T11 probe (129)
ctgctagttacctttg

SEQ ID NO: 69 - DNA, 15 bp, Artificial Sequence
  T13 probe (129)
aggaggaagacgcag

SEQ ID NO: 70 - DNA, 17 bp, Artificial Sequence
  T14 probe (129)
ctttgttcttcataagc

SEQ ID NO: 71 - DNA, 25 bp, Artificial Sequence
  C2 forward primer
atgagggatttccttaatcagacaa

SEQ ID NO: 72 - DNA, 29 bp, Artificial Sequence
  T3 forward primer
tggtatgtttattcttactcaaggttttg

SEQ ID NO: 73 - DNA, 22 bp, Artificial Sequence
  T6 forward primer
gggcaactgatggaaagaactc

SEQ ID NO: 74 - DNA, 23 bp, Artificial Sequence
  T7 forward primer
gactgacgcacaaacttgtcctt

SEQ ID NO: 75 - DNA, 26 bp, Artificial Sequence
  T8 forward primer
cccaaagcatataacaagaacaaatg

SEQ ID NO: 76 - DNA, 18 bp, Artificial Sequence
  T9 forward primer
gcaggacgcaggcgttta

SEQ ID NO: 77 - DNA, 23 bp, Artificial Sequence
  T10 forward primer
gcatcctcatggcagtctacatc

SEQ ID NO: 78 - DNA, 20 bp, Artificial Sequence
  T11 forward primer
cctgccccttgatgagtgtt

SEQ ID NO: 79 - DNA, 23 bp, Artificial Sequence
  T13 forward primer
ccctctttgatatgctcgtgtgt

SEQ ID NO: 80 - DNA, 22 bp, Artificial Sequence
  T14 forward primer
tcccacaggtccatgtctttaa

SEQ ID NO: 81 - DNA, 28 bp, Artificial Sequence
  C2 reverse primer
agactacaatgagctaccatcataaggt

SEQ ID NO: 82 - DNA, 24 bp, Artificial Sequence
  T3 reverse primer
caaccatctaaaactccagttcca

SEQ ID NO: 83 - DNA, 28 bp, Artificial Sequence
  T6 reverse primer
tgtgtaacaggacagttgaatgtagaga

SEQ ID NO: 84 - DNA, 19 bp, Artificial Sequence
  T7 reverse primer
cttaaaacccgccctgcat

SEQ ID NO: 85 - DNA, 26 bp, Artificial Sequence
  T8 reverse primer
ctacaggagatgtggctgttctatgt

SEQ ID NO: 86 - DNA, 22 bp, Artificial Sequence
  T9 reverse primer
tcagcgtgattcgcttgtagtc

SEQ ID NO: 87 - DNA, 26 bp, Artificial Sequence
  T10 reverse primer
tgcatagctgtttgaataatgacaag

SEQ ID NO: 88 - DNA, 21 bp, Artificial Sequence
  T11 reverse primer
tgcagcatctctgtcaagcaa

SEQ ID NO: 89 - DNA, 24 bp, Artificial Sequence
  T13 reverse primer
gcaacaacataacccacagcataa

SEQ ID NO: 90 - DNA, 23 bp, Artificial Sequence
  T14 reverse primer
gctaagcgtttggaagaaattcc

SEQ ID NO: 91 - DNA, 20 bp, Artificial Sequence
  SV 13.7 forward primer
taggctctaaggatgctggc

SEQ ID NO: 92 - DNA, 20 bp, Artificial Sequence
  SV 13.7 reverse primer
aagcagcttcaaaccctctg

SEQ ID NO: 93 - DNA, 20 bp, Artificial Sequence
  SV 20.0 forward primer
ttacttggccttggaactgc

SEQ ID NO: 94 - DNA, 21 bp, Artificial Sequence
  SV 20.0 reverse primer
tgattcgtaatcgtcactgcc

SEQ ID NO: 95 - DNA, 20 bp, Artificial Sequence
  SV 36.9 forward primer
tcctgtcccgagaaactgtc

SEQ ID NO: 96 - DNA, 20 bp, Artificial Sequence
  SV 36.9 reverse primer
agctggctttcagagagctg

SEQ ID NO: 97 - DNA, 20 bp, Artificial Sequence
  SV 56.7 forward primer
ttagaaagtgccaaccaggc

SEQ ID NO: 98 - DNA, 20 bp, Artificial Sequence
  SV 56.7 reverse primer
ctctggctaggaacaatggc

SEQ ID NO: 99 - DNA, 25 bp, Artificial Sequence
  m-lr-f primer
gttaggtgcagggtctactcagctg

SEQ ID NO: 100 - DNA, 20 bp, Artificial Sequence
  m-5'-f primer
ggaggagaggagaagcagcc

SEQ ID NO: 101 - DNA, 20 bp, Artificial Sequence
  m-A primer
ggaggagaggagaagcagcc

SEQ ID NO: 102 - DNA, 26 bp, Artificial Sequence
  h-lr-r primer
gcaaacagccttcttcccacattcgg

SEQ ID NO: 103 - DNA, 24 bp, Artificial Sequence
  m-5'-r primer
ttgctttcagtagttcaggtgtgc

SEQ ID NO: 104 - DNA, 20 bp, Artificial Sequence
  h-5'-r primer
ggcgttgtcaggaagttgcc

SEQ ID NO: 105 - DNA, 22 bp, Artificial Sequence
  m-F primer
tgaagttgagaggcacatgagg

SEQ ID NO: 106 - DNA, 24 bp, Artificial Sequence
  m-E2 primer
tagagtagccacaggcagcaaagc

SEQ ID NO: 107 - RNA, 21 nt, Artificial Sequence
  Cmah gRNA A DNA-targeting segment
gugacaggaaggcuucucacc

SEQ ID NO: 108 - RNA, 21 nt, Artificial Sequence
  Cmah gRNA B DNA-targeting segment
gcuuacaagcaauuugcugac

SEQ ID NO: 109 - DNA, 108 bp, Artificial Sequence
  Cmah locus
ttgccagtgaccctgtttgcagttagagttgacaggaaggcttctcacccgggacattttaaatgacccagtcagcaaattgcttgtaagttttggtgttctttcatt

SEQ ID NO: 110 - DNA, 46 bp, Artificial Sequence
  Cmah locus upstream of gRNA A cut
ttgccagtgaccctgtttgcagttagagttgacaggaaggcttctc

SEQ ID NO: 111 - DNA, 35 bp, Artificial Sequence
  Cmah locus downstream of gRNA B cut
agcaaattgcttgtaagttttggtgttctttcatt

SEQ ID NO: 112 - DNA, 27 bp, Artificial Sequence
  Cmah locus sequence excised by gRNAs A and B
acccgggacattttaaatgacccagtc

SEQ ID NO: 113 - DNA, 21 bp, Artificial Sequence
  C5 primer m-5'-F
accccagcatctgacgacacc

SEQ ID NO: 114 - DNA, 20 bp, Artificial Sequence
  C5 primer m-5'-R
agaaagaccgcagtggaacc

SEQ ID NO: 115 - DNA, 21 bp, Artificial Sequence
  C5 primer h-5'-R
tccccacatgcctagtaggag

SEQ ID NO: 116 - DNA, 22 bp, Artificial Sequence
  Cmah TaqMan forward primer
gtgaccctgtttgcagttagag

SEQ ID NO: 117 - DNA, 23 bp, Artificial Sequence
  Cmah TaqMan probe
acaggaaggcttctcacccggga

SEQ ID NO: 118 - DNA, 24 bp, Artificial Sequence
  Cmah TaqMan reverse primer
tgaagtcaggaaactgttccaatg

SEQ ID NO: 119 - DNA, 22 bp, Artificial Sequence
  7064retU forward primer
cctcctgagctttcctttgcag

SEQ ID NO: 120 - DNA, 25 bp, Artificial Sequence
  7064retU reverse primer
cctagacaacacagacactgtatca

SEQ ID NO: 121 - DNA, 23 bp, Artificial Sequence
  7064retU TaqMan probe
ttctgcccttgaaaaggagaggc

SEQ ID NO: 122 - DNA, 18 bp, Artificial Sequence
  7064retD forward primer
cctctgaggccacctgaa

SEQ ID NO: 123 - DNA, 23 bp, Artificial Sequence
  7064retD reverse primer
ccctgacaagttctgccttctac

SEQ ID NO: 124 - DNA, 21 bp, Artificial Sequence
  7064retD TaqMan probe
tgcccaagcctctgcagcttt

SEQ ID NO: 125 - DNA, 19 bp, Artificial Sequence
  7140retU forward primer
cccagcatctgacgacacc

SEQ ID NO: 126 - DNA, 21 bp, Artificial Sequence
  7140retU reverse primer
gaccactgtgggcatctgtag

SEQ ID NO: 127 - DNA, 27 bp, Artificial Sequence
  7140retU TaqMan probe
ccgagtctgctgttactgttagcatca

SEQ ID NO: 128 - DNA, 20 bp, Artificial Sequence
  7140retD forward primer
cccgacaccttctgagcatg

SEQ ID NO: 129 - DNA, 21 bp, Artificial Sequence
  7140retD reverse primer
tgcaggctgagtcaggatttg

SEQ ID NO: 130 - DNA, 25 bp, Artificial Sequence
  7140retD TaqMan probe
tagtcacgttttgtgacaccccaga

SEQ ID NO: 131 - DNA, 22 bp, Artificial Sequence
  mADAM6-2 LOA forward primer
agggctgagggagaacatatac

SEQ ID NO: 132 - DNA, 20 bp, Artificial Sequence
  mADAM6-2 LOA reverse primer
aggcctgatgcaggagctat

SEQ ID NO: 133 - DNA, 26 bp, Artificial Sequence
  mADAM6-2 LOA probe
tcctctcagctggattaacagcatca

SEQ ID NO: 134 - DNA, 20 bp, Artificial Sequence
  hIgH31 LOA forward primer
atcacactcatcccatcccc

SEQ ID NO: 135 - DNA, 20 bp, Artificial Sequence
  hIgH31 LOA reverse primer
cacagggaagcaggaactgc

SEQ ID NO: 136 - DNA, 29 bp, Artificial Sequence
  hIgH31 LOA probe
cccttccctaagtaccacagagtgggctc

SEQ ID NO: 137 - DNA, 19 bp, Artificial Sequence
  hIgH9 LOA forward primer
tcctccaacgacaggtccc

SEQ ID NO: 138 - DNA, 20 bp, Artificial Sequence
  hIgH9 LOA reverse primer
gatgaactgacgggcacagg

SEQ ID NO: 139 - DNA, 24 bp, Artificial Sequence
  hIgH9 LOA probe
tccctggaactctgccccgacaca

SEQ ID NO: 140 - DNA, 19 bp, Artificial Sequence
  hIgH1 LOA forward primer
cagtcccgttgatccagcc

SEQ ID NO: 141 - DNA, 21 bp, Artificial Sequence
  hIgH1 LOA reverse primer
ggatatgcagcactgtgccac

SEQ ID NO: 142 - DNA, 30 bp, Artificial Sequence
  hIgH1 LOA probe
cccatcagggattttgtatctctgtggacg

SEQ ID NO: 143 - DNA, 19 bp, Artificial Sequence
  Neo GOA forward primer
ggtggagaggctattcggc

SEQ ID NO: 144 - DNA, 17 bp, Artificial Sequence
  Neo GOA reverse primer
gaacacggcggcatcag

SEQ ID NO: 145 - DNA, 23 bp, Artificial Sequence
  Neo GOA probe
tgggcacaacagacaatcggctg

SEQ ID NO: 146 - DNA, 19 bp, Artificial Sequence
  5' IgH Arm1 retention assay forward primer
aggatgctgggaaacagac

SEQ ID NO: 147 - DNA, 20 bp, Artificial Sequence
  5' IgH Arm1 retention assay reverse primer
gaccactctcaggactctca

SEQ ID NO: 148 - DNA, 24 bp, Artificial Sequence
  5' IgH Arm1 retention assay probe
tggaaggtcccaaaggaaaccaca

SEQ ID NO: 149 - DNA, 22 bp, Artificial Sequence
  mIgM398 retention assay forward primer
gagctcacaccttgacctttca

SEQ ID NO: 150 - DNA, 22 bp, Artificial Sequence
  mIgM398 retention assay reverse primer
tggtgggacgaacacatttaca

SEQ ID NO: 151 - DNA, 24 bp, Artificial Sequence
  mIgM398 retention assay probe
ccagctgtcgcagagatgaacccc

SEQ ID NO: 152 - DNA, 22 bp, Artificial Sequence
  mIgM1045 retention assay forward primer
tccctccacagacatcctaacc

SEQ ID NO: 153 - DNA, 21 bp, Artificial Sequence
  mIgM1045 retention assay reverse primer
gttagcggacttgctgaggaa

SEQ ID NO: 154 - DNA, 22 bp, Artificial Sequence
  mIgM1045 retention assay probe
tcaccatccccccctcctttgc

SEQ ID NO: 155 - DNA, 22 bp, Artificial Sequence
  3' IgH Arm2 retention assay forward primer
ggtcatgtggcaaggctatttg

SEQ ID NO: 156 - DNA, 21 bp, Artificial Sequence
  3' IgH Arm2 retention assay reverse primer
agcctggactttcggtttggt

SEQ ID NO: 157 - DNA, 30 bp, Artificial Sequence
  3' IgH Arm2 retention assay probe
ccactaggtaaacttgtagctgtggtttga

SEQ ID NO: 158 - DNA, 17 bp, Artificial Sequence
  mIgHp2 parental forward primer
gccatgcaaggccaagc

SEQ ID NO: 159 - DNA, 24 bp, Artificial Sequence
  mIgHp2 parental reverse primer
agttcttgagccttagggtgctag

SEQ ID NO: 160 - DNA, 24 bp, Artificial Sequence
  mIgHp2 parental probe
ccaggaaaatgctgccagagcctg

SEQ ID NO: 161 - DNA, 20 bp, Artificial Sequence
  mIgKd2 parental forward primer
gcaaacaaaaaccactggcc

SEQ ID NO: 162 - DNA, 19 bp, Artificial Sequence
  mIgKd2 parental reverse primer
ggccacattccatgggttc

SEQ ID NO: 163 - DNA, 37 bp, Artificial Sequence
  mIgKd2 parental probe
ctgttcctctaaaactggactccacagtaaatggaaa

SEQ ID NO: 164 - DNA, 20 bp, Artificial Sequence
  hIgK5 parental forward primer
ccccgtcctcctcctttttc

SEQ ID NO: 165 - DNA, 19 bp, Artificial Sequence
  hIgK5 parental reverse primer
tgcaagtgctgccagcaag

SEQ ID NO: 166 - DNA, 32 bp, Artificial Sequence
  hIgK5 parental probe
tcatgtccattaacccatttaccttttgccca

SEQ ID NO: 167 - DNA, 21 bp, Artificial Sequence
  3' gRNA_I DNA-targeting sequence
gactactacggtatggacgtc

SEQ ID NO: 168 - DNA, 21 bp, Artificial Sequence
  3' gRNA_II DNA-targeting sequence
gctactacggtatggacgtct

SEQ ID NO: 169 - DNA, 20 bp, Artificial Sequence
  5' gRNA_I DNA-targeting sequence
gaagctgactagtttacgca

SEQ ID NO: 170 - DNA, 21 bp, Artificial Sequence
  5' gRNA_II DNA-targeting sequence
gtagcattcttacacctagca

SEQ ID NO: 171 - DNA, 23 bp, Artificial Sequence
  5' IgH Arm2 retention assay forward primer
ctgagcatactgctgcctaacac

SEQ ID NO: 172 - DNA, 25 bp, Artificial Sequence
  5' IgH Arm2 retention assay reverse primer
gagcagtgcatttcttagttaagga

SEQ ID NO: 173 - DNA, 26 bp, Artificial Sequence
  5' IgH Arm2 retention assay probe
tgaaatggcagttcttctccagctgg

SEQ ID NO: 174 - DNA, 20 bp, Artificial Sequence
  3' IgH Arm1 retention assay forward primer
ggtggagtccctggatgatg

SEQ ID NO: 175 - DNA, 21 bp, Artificial Sequence
  3' IgH Arm1 retention assay reverse primer
atccctccagccataggattg

SEQ ID NO: 176 - DNA, 28 bp, Artificial Sequence
  3' IgH Arm1 retention assay probe
ctttggaggctcatttgagggagatgct